European Patent Application EP 4 756 428 A1, published June 10, 2026. Title: Hydrogel-based polymeric 3D-scaffold for detecting the viability of cells. Applicant: Universität Heidelberg. The sequence listing filed with the application follows.

SEQUENCE LISTING (26 sequences)

SEQ ID NO: 1 - skipped

SEQ ID NO: 2 - protein, 4 aa, synthetic construct
  source 1..4: note = caspase-cleavable peptide
DEVD

SEQ ID NO: 3 - protein, 4 aa, synthetic construct
  source 1..4: note = caspase-cleavable peptide
VEID

SEQ ID NO: 4 - protein, 4 aa, synthetic construct
  source 1..4: note = caspase-cleavable peptide
IETD

SEQ ID NO: 5 - protein, 4 aa, synthetic construct
  source 1..4: note = caspase-cleavable peptide
LEHD

SEQ ID NO: 6 - protein, 6 aa, synthetic construct
  source 1..6: note = caspase-cleavable peptide
  VARIANT 1
  VARIANT 6
XDEVDX

SEQ ID NO: 7 - protein, 6 aa, synthetic construct
  source 1..6: note = caspase-cleavable peptide
DDEVDK

SEQ ID NO: 8 - protein, 15 aa, synthetic construct
  source 1..15: note = peptide mediating cell-matrix attachment
GFOGERGVEGPOGPA

SEQ ID NO: 9 - protein, 5 aa, synthetic construct
  source 1..5: note = peptide mediating cell-matrix attachment
LPGER

SEQ ID NO: 10 - protein, 6 aa, synthetic construct
  source 1..6: note = peptide mediating cell-matrix attachment
GLPGER

SEQ ID NO: 11 - protein, 6 aa, synthetic construct
  source 1..6: note = peptide mediating cell-matrix attachment
  VARIANT 2
GXOGER

SEQ ID NO: 12 - protein, 5 aa, synthetic construct
  source 1..5: note = peptide mediating cell-matrix attachment
GFOGE

SEQ ID NO: 13 - protein, 9 aa, synthetic construct
  source 1..9: note = peptide mediating cell-matrix attachment
CDPGYIGSR

SEQ ID NO: 14 - protein, 15 aa, synthetic construct
  source 1..15: note = peptide comprising extracellular matrix (ECM) protein-binding domain
  VARIANT 3
  VARIANT 4
IQNNKFEYKEDTIKE

SEQ ID NO: 15 - protein, 7 aa, synthetic construct
  source 1..7: note = peptide comprising extracellular matrix (ECM) protein-binding domain
TKKTLRT

SEQ ID NO: 16 - protein, 9 aa, synthetic construct
  source 1..9: note = peptide comprising extracellular matrix (ECM) protein-binding domain
  VARIANT 7
  VARIANT 8
  VARIANT 9
LRELHLNNN

SEQ ID NO: 17-18 - skipped (2 entries)

SEQ ID NO: 19 - protein, 10 aa, synthetic construct
  source 1..10: note = peptide comprising a domain being recognized by a metalloproteinase
ALRRLLGLFG

SEQ ID NO: 20 - protein, 9 aa, synthetic construct
  source 1..9: note = peptide comprising a domain being recognized by a metalloproteinase
ALRRLLSLF

SEQ ID NO: 21-22 - skipped (2 entries)

SEQ ID NO: 23 - protein, 6 aa, synthetic construct
  source 1..6: note = peptide comprising a domain being recognized by a metalloproteinase
PVPQGS

SEQ ID NO: 24 - protein, 26 aa, synthetic construct
  source 1..26: note = peptide comprising a domain for a growth factor
MTAASMGPVRVAFVVLLALCSRPAVG

SEQ ID NO: 25 - protein, 14 aa, synthetic construct
  source 1..14: note = peptide comprising a domain for a growth factor
DYLAGFKAHGKKYR

SEQ ID NO: 26 - protein, 5 aa, synthetic construct
  source 1..5: note = peptide comprising a domain for a growth factor
CTCCC